European Patent Application EP 4 740 967 A1, published May 13, 2026. Title: 一种连接子-药物分子及抗体药物偶联物、其制备方法和应用. Applicant: 上海诗健生物科技有限公司. The sequence listing filed with the application follows.

SEQUENCE LISTING (4 sequences)

SEQ ID NO: 1 - protein, 447 aa, synthetic construct
QIQLVQSGAEVKKPGASVKISCKASGYSFTDYHMNWVRQAPGKGLEWIGNIDPYYGSPTYNHKFKGRVTLTVDTSTSTAYMELSSLRSEDTAVYYCANYGRGNSFPYWGQGTLVTVSSASTKGPSVFPLAPSSKSTSGGTAALGCLVKDYFPEPVTVSWNSGALTSGVHTFPAVLQSSGLYSLSSVVTVPSSSLGTQTYICNVNHKPSNTKVDKKVEPKSCDKTHTCPPCPAPELLGGPSVFLFPPKPKDTLMISRTPEVTCVVVDVSHEDPEVKFNWYVDGVEVHNAKTKPREEQYNSTYRVVSVLTVLHQDWLNGKEYKCKVSNKALPAPIEKTISKAKGQPREPQVYTLPPSRDELTKNQVSLTCLVKGFYPSDIAVEWESNGQPENNYKTTPPVLDSDGSFFLYSKLTVDKSRWQQGNVFSCSVMHEALHNHYTQKSLSLSPG

SEQ ID NO: 2 - protein, 220 aa, synthetic construct
DIVMTQSPSSLAVSLGERATINCKSSQSLLNSGNQRNYLTWYQQKPGQPPKLLIYWASTRESGVPDRFSGSGSGTDFTLTISSLQAEDVAVYYCQNDYSFPFTFGQGTKLEIKRTVAAPSVFIFPPSDEQLKSGTASVVCLLNNFYPREAKVQWKVDNALQSGNSQESVTEQDSKDSTYSLSSTLTLSKADYEKHKVYACEVTHQGLSSPVTKSFNRGEC

SEQ ID NO: 3 - protein, 449 aa, synthetic construct
EVQLVESGGGVVQPGRSLRLSCSASGFTFSGYGLSWVRQAPGKGLEWVAMISSGGSYTYYADSVKGRFAISRDNAKNTLFLQMDSLRPEDTGVYFCARHGDDPAWFAYWGQGTPVTVSSASTKGPSVFPLAPSSKSTSGGTAALGCLVKDYFPEPVTVSWNSGALTSGVHTFPAVLQSSGLYSLSSVVTVPSSSLGTQTYICNVNHKPSNTKVDKKVEPKSCDKTHTCPPCPAPELLGGPSVFLFPPKPKDTLMISRTPEVTCVVVDVSHEDPEVKFNWYVDGVEVHNAKTKPREEQYNSTYRVVSVLTVLHQDWLNGKEYKCKVSNKALPAPIEKTISKAKGQPREPQVYTLPPSRDELTKNQVSLTCLVKGFYPSDIAVEWESNGQPENNYKTTPPVLDSDGSFFLYSKLTVDKSRWQQGNVFSCSVMHEALHNHYTQKSLSLSPGK

SEQ ID NO: 4 - protein, 217 aa, synthetic construct
DIQLTQSPSSLSASVGDRVTITCSVSSSISSNNLHWYQQKPGKAPKPWIYGTSNLASGVPSRFSGSGSGTDYTFTISSLQPEDIATYYCQQWSSYPYMYTFGQGTKVEIKRTVAAPSVFIFPPSDEQLKSGTASVVCLLNNFYPREAKVQWKVDNALQSGNSQESVTEQDSKDSTYSLSSTLTLSKADYEKHKVYACEVTHQGLSSPVTKSFNRGEC